European Patent Application EP 4 273 175 A1, published November 8, 2023. Title: Novel chimeric antigen receptor and use thereof. Applicant: Bioheng Therapeutics Limited. The sequence listing filed with the application follows.

SEQUENCE LISTING (83 sequences)

SEQ ID NO: 1 - protein, 11 aa, Artificial Sequence
  CD7 scFv CDR-L1
RASQSISNNLH

SEQ ID NO: 2 - protein, 7 aa, Artificial Sequence
  CD7 scFv CDR-L2
SASQSIS

SEQ ID NO: 3 - protein, 9 aa, Artificial Sequence
  CD7 scFv CDR-L3
QQSNSWPYT

SEQ ID NO: 4 - protein, 7 aa, Artificial Sequence
  CD7 scFv CDR-H1
GYTFTSY

SEQ ID NO: 5 - protein, 6 aa, Artificial Sequence
  CD7 scFv CDR-H2
NPSNGR

SEQ ID NO: 6 - protein, 14 aa, Artificial Sequence
  CD7 scFv CDR-H3
GGVYYDLYYYALDY

SEQ ID NO: 7 - protein, 108 aa, Artificial Sequence
  m189 VL
DIELTQSPATLSVTPGDSVSLSCRASQSISNNLHWYQQKSHESPRLLIKSASQSISGIPSRFSGSGSGTDFTLSINSVETEDFGMYFCQQSNSWPYTFGGGTKLEIKR

SEQ ID NO: 8 - protein, 123 aa, Artificial Sequence
  m189 VH
QVQLQESGAELVKPGASVKLSCKASGYTFTSYWMHWVKQRPGQGLEWIGKINPSNGRTNYNEKFKSKATLTVDKSSSTAYMQLSSLTSEDSAVYYCARGGVYYDLYYYALDYWGQGTTVTVSS

SEQ ID NO: 9 - protein, 249 aa, Artificial Sequence
  m189 scFv
DIELTQSPATLSVTPGDSVSLSCRASQSISNNLHWYQQKSHESPRLLIKSASQSISGIPSRFSGSGSGTDFTLSINSVETEDFGMYFCQQSNSWPYTFGGGTKLEIKRGSTSGSGKPGSGEGSTKGQVQLQESGAELVKPGASVKLSCKASGYTFTSYWMHWVKQRPGQGLEWIGKINPSNGRTNYNEKFKSKATLTVDKSSSTAYMQLSSLTSEDSAVYYCARGGVYYDLYYYALDYWGQGTTVTVSS

SEQ ID NO: 10 - protein, 108 aa, Artificial Sequence
  h189-1 VL
EIVLTQSPATLSLSPGERATLSCRASQSISNNLHWYQQKPGQAPRLLIYSASQSISGIPARFSGSGPGTDFTLTISSLEPEDFAVYYCQQSNSWPYTFGQGTKVEIKR

SEQ ID NO: 11 - protein, 123 aa, Artificial Sequence
  h189-1 VH
QVQLVQSGAEVKKPGASVKVSCKASGYTFTSYYMHWVRQAPGQGLEWMGWINPSNGRTNYAQKFQGRVTMTRDTSISTAYMELSRLRSDDTAVYYCARGGVYYDLYYYALDYWGQGTLVTVSS

SEQ ID NO: 12 - protein, 249 aa, Artificial Sequence
  h189-1 scFv
EIVLTQSPATLSLSPGERATLSCRASQSISNNLHWYQQKPGQAPRLLIYSASQSISGIPARFSGSGPGTDFTLTISSLEPEDFAVYYCQQSNSWPYTFGQGTKVEIKRGSTSGSGKPGSGEGSTKGQVQLVQSGAEVKKPGASVKVSCKASGYTFTSYYMHWVRQAPGQGLEWMGWINPSNGRTNYAQKFQGRVTMTRDTSISTAYMELSRLRSDDTAVYYCARGGVYYDLYYYALDYWGQGTLVTVSS

SEQ ID NO: 13 - protein, 108 aa, Artificial Sequence
  h189-2 VL
DVVMTQSPAFLSVTPGEKVTITCRASQSISNNLHWYQQKPDQAPKLLIKSASQSISGVPSRFSGSGSGTDFTFTISSLEAEDAATYYCQQSNSWPYTFGQGTKVEIKR

SEQ ID NO: 14 - protein, 123 aa, Artificial Sequence; identical to SEQ ID NO: 11
  h189-2 VH

SEQ ID NO: 15 - protein, 249 aa, Artificial Sequence
  h189-2 scFv
DVVMTQSPAFLSVTPGEKVTITCRASQSISNNLHWYQQKPDQAPKLLIKSASQSISGVPSRFSGSGSGTDFTFTISSLEAEDAATYYCQQSNSWPYTFGQGTKVEIKRGSTSGSGKPGSGEGSTKGQVQLVQSGAEVKKPGASVKVSCKASGYTFTSYYMHWVRQAPGQGLEWMGWINPSNGRTNYAQKFQGRVTMTRDTSISTAYMELSRLRSDDTAVYYCARGGVYYDLYYYALDYWGQGTLVTVSS

SEQ ID NO: 16 - protein, 108 aa, Artificial Sequence
  h189-3 VL
DVVMTQSPAFLSVTPGEKVTITCRASQSISNNLHWYQQKPDQAPKLLIKSASQSISGVPSRFSGSGSGTDFTFTISSLEAEDAAMYFCQQSNSWPYTFGQGTKVEIKR

SEQ ID NO: 17 - protein, 123 aa, Artificial Sequence
  h189-3 VH
QVQLVQSGAEVKKPGASVKVSCKASGYTFTSYWMHWVRQAPGQGLEWMGKINPSNGRTNYAQKFQGRVTMTRDTSISTAYMELSRLRSDDTAVYYCARGGVYYDLYYYALDYWGQGTLVTVSS

SEQ ID NO: 18 - protein, 249 aa, Artificial Sequence
  h189-3 scFv
DVVMTQSPAFLSVTPGEKVTITCRASQSISNNLHWYQQKPDQAPKLLIKSASQSISGVPSRFSGSGSGTDFTFTISSLEAEDAAMYFCQQSNSWPYTFGQGTKVEIKRGSTSGSGKPGSGEGSTKGQVQLVQSGAEVKKPGASVKVSCKASGYTFTSYWMHWVRQAPGQGLEWMGKINPSNGRTNYAQKFQGRVTMTRDTSISTAYMELSRLRSDDTAVYYCARGGVYYDLYYYALDYWGQGTLVTVSS

SEQ ID NO: 19 - protein, 108 aa, Artificial Sequence
  h189-4 VL
EIVLTQSPATLSLSPGERATLSCRASQSISNNLHWYQQKPGQAPRLLIKSASQSISGIPARFSGSGPGTDFTLTISSLEPEDFAVYFCQQSNSWPYTFGQGTKVEIKR

SEQ ID NO: 20 - protein, 123 aa, Artificial Sequence; identical to SEQ ID NO: 17
  h189-4 VH

SEQ ID NO: 21 - protein, 249 aa, Artificial Sequence
  h189-4 scFv
EIVLTQSPATLSLSPGERATLSCRASQSISNNLHWYQQKPGQAPRLLIKSASQSISGIPARFSGSGPGTDFTLTISSLEPEDFAVYFCQQSNSWPYTFGQGTKVEIKRGSTSGSGKPGSGEGSTKGQVQLVQSGAEVKKPGASVKVSCKASGYTFTSYWMHWVRQAPGQGLEWMGKINPSNGRTNYAQKFQGRVTMTRDTSISTAYMELSRLRSDDTAVYYCARGGVYYDLYYYALDYWGQGTLVTVSS

SEQ ID NO: 22 - protein, 25 aa, Artificial Sequence
  CD8alpha transmembrane domain
IYIWAPLAGTCGVLLLSLVITLYCK

SEQ ID NO: 23 - DNA, 75 bp, Artificial Sequence
  CD8alpha transmembrane domain
atctacatctgggcgcccttggccgggacttgtggggtccttctcctgtcactggttatcaccctttactgcaaa

SEQ ID NO: 24 - protein, 27 aa, Artificial Sequence
  CD28 transmembrane domain
FWVLVVVGGVLACYSLLVTVAFIIFWV

SEQ ID NO: 25 - DNA, 81 bp, Artificial Sequence
  CD28 transmembrane domain
ttttgggtcctcgtcgtagttggaggggtacttgcctgttatagcctcctggttaccgtagcatttattatattctgggtg

SEQ ID NO: 26 - protein, 41 aa, Artificial Sequence
  CD28 costimulatory domain
RSKRSRLLHSDYMNMTPRRPGPTRKHYQPYAPPRDFAAYRS

SEQ ID NO: 27 - DNA, 123 bp, Artificial Sequence
  CD28 costimulatory domain
aggagtaagaggagcaggctcctgcacagtgactacatgaacatgactccccgccgccccgggcccacccgcaagcattaccagccctatgccccaccacgcgacttcgcagcctatcgctcc

SEQ ID NO: 28 - protein, 40 aa, Artificial Sequence
  4-1BB costimulatory domain
RGRKKLLYIFKQPFMRPVQTTQEEDGCSCRFPEEEEGGCE

SEQ ID NO: 29 - DNA, 120 bp, Artificial Sequence
  4-1BB costimulatory domain
cggggcagaaagaaactcctgtatatattcaaacaaccatttatgagaccagtacaaactactcaagaggaagatggctgtagctgccgatttccagaagaagaagaaggaggatgtgaa

SEQ ID NO: 30 - protein, 113 aa, Artificial Sequence
  CD3zeta signaling domain
LRVKFSRSADAPAYQQGQNQLYNELNLGRREEYDVLDKRRGRDPEMGGKPRRKNPQEGLYNELQKDKMAEAYSEIGMKGERRRGKGHDGLYQGLSTATKDTYDALHMQALPPR

SEQ ID NO: 31 - DNA, 339 bp, Artificial Sequence
  CD3zeta signaling domain
ctgagagtgaagttcagcaggagcgcagacgcccccgcgtaccagcagggccagaaccagctctataacgagctcaatctaggacgaagagaggagtacgatgttttggacaagagacgtggccgggaccctgagatggggggaaagccgagaaggaagaaccctcaggaaggcctgtacaatgaactgcagaaagataagatggcggaggcctacagtgagattgggatgaaaggcgagcgccggaggggcaaggggcacgatggcctttaccagggtctcagtacagccaccaaggacacctacgacgcccttcacatgcaggccctgccccctcgc

SEQ ID NO: 32 - protein, 114 aa, Artificial Sequence
  CD3zeta signaling domain
LRVKFSRSADAPAYQQGQNQLFNELNLGRREEFDVLDKRRGRDPEMGGKPQRRKNPQEGLYNELQKDKMAEAYSEIGMKGERRRGKGHDGLFQGLSTATKDTFDALHMQALPPR

SEQ ID NO: 33 - DNA, 342 bp, Artificial Sequence
  CD3zeta signaling domain
ctgagagtgaagttcagcaggagcgcagacgcccccgcgtaccagcagggccagaaccagctctttaacgagctcaatctaggacgaagagaggagttcgatgttttggacaagagacgtggccgggaccctgagatggggggaaagccgcagagaaggaagaaccctcaggaaggcctgtacaatgaactgcagaaagataagatggcggaggcctacagtgagattgggatgaaaggcgagcgccggaggggcaaggggcacgatggccttttccagggtctcagtacagccaccaaggacacctttgacgcccttcacatgcaggccctgccccctcgc

SEQ ID NO: 34 - protein, 20 aa, Artificial Sequence
  B2M signal peptide
MSRSVALAVLALLSLSGLEA

SEQ ID NO: 35 - DNA, 60 bp, Artificial Sequence
  B2M signal domain
atgtcccgctctgttgctttggctgtgctggcccttttgtcccttagcggactggaggcc

SEQ ID NO: 36 - protein, 21 aa, Artificial Sequence
  CD8alpha signal peptide
MALPVTALLLPLALLLHAARP

SEQ ID NO: 37 - DNA, 63 bp, Artificial Sequence
  CD8alpha signal peptide
atggccttaccagtgaccgccttgctcctgccgctggccttgctgctccacgccgccaggccg

SEQ ID NO: 38 - protein, 45 aa, Artificial Sequence
  CD8alpha hinge region
TTTPAPRPPTPAPTIASQPLSLRPEACRPAAGGAVHTRGLDFACD

SEQ ID NO: 39 - DNA, 135 bp, Artificial Sequence
  CD8alpha hinge region
accacgacgccagcgccgcgaccaccaacaccggcgcccaccatcgcgtcgcagcccctgtccctgcgcccagaggcgtgccggccagcggcggggggcgcagtgcacacgagggggctggacttcgcctgtgat

SEQ ID NO: 40 - protein, 39 aa, Artificial Sequence
  CD28 hinge region
IEVMYPPPYLDNEKSNGTIIHVKGKHLCPSPLFPGPSKP

SEQ ID NO: 41 - DNA, 117 bp, Artificial Sequence
  CD28 hinge region
attgaagttatgtatcctcctccttacctagacaatgagaagagcaatggaaccattatccatgtgaaagggaaacacctttgtccaagtcccctatttcccggaccttctaagccc

SEQ ID NO: 42 - protein, 12 aa, Artificial Sequence
  IgG4 hinge region
ESKYGPPCPPCP

SEQ ID NO: 43 - DNA, 36 bp, Artificial Sequence
  IgG4 hinge region
gaaagcaaatacgggccgccgtgtccaccctgtccg

SEQ ID NO: 44 - protein, 11 aa, Artificial Sequence
  CD19 scFv-1 CDR-L1
RASQDISKYLN

SEQ ID NO: 45 - protein, 7 aa, Artificial Sequence
  CD19 scFv-1 CDR-L2
HTSRLHS

SEQ ID NO: 46 - protein, 9 aa, Artificial Sequence
  CD19 scFv-1 CDR-L3
QQGNTLPYT

SEQ ID NO: 47 - protein, 7 aa, Artificial Sequence
  CD19 scFv-1 CDR-H1
GVSLPDY

SEQ ID NO: 48 - protein, 5 aa, Artificial Sequence
  CD19 scFv-1 CDR-H2
WGSET

SEQ ID NO: 49 - protein, 12 aa, Artificial Sequence
  CD19 scFv-1 CDR-H3
HYYYGGSYAMDY

SEQ ID NO: 50 - protein, 11 aa, Artificial Sequence
  CD19 scFv-2 CDR-L1
QASEDIYSGLA

SEQ ID NO: 51 - protein, 7 aa, Artificial Sequence
  CD19 scFv-2 CDR-L2
GASDLQD

SEQ ID NO: 52 - protein, 9 aa, Artificial Sequence
  CD19 scFv-2 CDR-L3
QQGLTYPRT

SEQ ID NO: 53 - protein, 7 aa, Artificial Sequence
  CD19 scFv-2 CDR-H1
GDTITFY

SEQ ID NO: 54 - protein, 6 aa, Artificial Sequence
  CD19 scFv-2 CDR-H2
DPEDES

SEQ ID NO: 55 - protein, 7 aa, Artificial Sequence
  CD19 scFv-2 CDR-H3
GGYYFDY

SEQ ID NO: 56 - protein, 107 aa, Artificial Sequence
  CD19 scFv-1 VL
DIQMTQTTSSLSASLGDRVTISCRASQDISKYLNWYQQKPDGTVKLLIYHTSRLHSGVPSRFSGSGSGTDYSLTISNLEQEDIATYFCQQGNTLPYTFGGGTKLEIT

SEQ ID NO: 57 - protein, 120 aa, Artificial Sequence
  CD19 scFv-1 VH
EVKLQESGPGLVAPSQSLSVTCTVSGVSLPDYGVSWIRQPPRKGLEWLGVIWGSETTYYNSALKSRLTIIKDNSKSQVFLKMNSLQTDDTAIYYCAKHYYYGGSYAMDYWGQGTSVTVSS

SEQ ID NO: 58 - protein, 242 aa, Artificial Sequence
  CD19 scFv-1
DIQMTQTTSSLSASLGDRVTISCRASQDISKYLNWYQQKPDGTVKLLIYHTSRLHSGVPSRFSGSGSGTDYSLTISNLEQEDIATYFCQQGNTLPYTFGGGTKLEITGGGGSGGGGSGGGGSEVKLQESGPGLVAPSQSLSVTCTVSGVSLPDYGVSWIRQPPRKGLEWLGVIWGSETTYYNSALKSRLTIIKDNSKSQVFLKMNSLQTDDTAIYYCAKHYYYGGSYAMDYWGQGTSVTVSS

SEQ ID NO: 59 - protein, 107 aa, Artificial Sequence
  CD19 scFv-2 VL
DIQMTQSPASLSTSLGETVTIQCQASEDIYSGLAWYQQKPGKSPQLLIYGASDLQDGVPSRFSGSGSGTQYSLKITSMQTEDEGVYFCQQGLTYPRTFGGGTKLELK

SEQ ID NO: 60 - protein, 116 aa, Artificial Sequence
  CD19 scFv-2 VH
EVQLQQSGAELVRPGTSVKLSCKVSGDTITFYYMHFVKQRPGQGLEWIGRIDPEDESTKYSEKFKNKATLTADTSSNTAYLKLSSLTSEDTATYFCIYGGYYFDYWGQGVMVTVSS

SEQ ID NO: 61 - protein, 238 aa, Artificial Sequence
  CD19 scFv-2
DIQMTQSPASLSTSLGETVTIQCQASEDIYSGLAWYQQKPGKSPQLLIYGASDLQDGVPSRFSGSGSGTQYSLKITSMQTEDEGVYFCQQGLTYPRTFGGGTKLELKGGGGSGGGGSGGGGSEVQLQQSGAELVRPGTSVKLSCKVSGDTITFYYMHFVKQRPGQGLEWIGRIDPEDESTKYSEKFKNKATLTADTSSNTAYLKLSSLTSEDTATYFCIYGGYYFDYWGQGVMVTVSS

SEQ ID NO: 62 - DNA, 1107 bp, Artificial Sequence
  gamma chain
atgttgaagccatcattaccattcacatccctcttattcctgcagctgcccctgctgggagtggggctgaacacgacaattctgacgcccaatgggaatgaagacaccacagctgatttcttcctgaccactatgcccactgactccctcagtgtttccactctgcccctcccagaggttcagtgttttgtgttcaatgtcgagtacatgaattgcacttggaacagcagctctgagccccagcctaccaacctcactctgcattattggtacaagaactcggataatgataaagtccagaagtgcagccactatctattctctgaagaaatcacttctggctgtcagttgcaaaaaaaggagatccacctctaccaaacatttgttgttcagctccaggacccacgggaacccaggagacaggccacacagatgctaaaactgcagaatctggtgatcccctgggctccagagaacctaacacttcacaaactgagtgaatcccagctagaactgaactggaacaacagattcttgaaccactgtttggagcacttggtgcagtaccggactgactgggaccacagctggactgaacaatcagtggattatagacataagttctccttgcctagtgtggatgggcagaaacgctacacgtttcgtgttcggagccgctttaacccactctgtggaagtgctcagcattggagtgaatggagccacccaatccactgggggagcaatacttcaaaagagaatcctttcctgtttgcattggaagccgtggttatctctgttggctccatgggattgattatcagccttctctgtgtgtatttctggctggaacggacgatgccccgaattcccaccctgaagaacctagaggatcttgttactgaataccacgggaacttttcggcctggagtggtgtgtctaagggactggctgagagtctgcagccagactacagtgaacgactctgcctcgtcagtgagattcccccaaaaggaggggcccttggggaggggcctggggcctccccatgcaaccagcatagcccctactgggcccccccatgttacaccctaaagcctgaaacc

SEQ ID NO: 63 - protein, 369 aa, Artificial Sequence
  gamma chain
MLKPSLPFTSLLFLQLPLLGVGLNTTILTPNGNEDTTADFFLTTMPTDSLSVSTLPLPEVQCFVFNVEYMNCTWNSSSEPQPTNLTLHYWYKNSDNDKVQKCSHYLFSEEITSGCQLQKKEIHLYQTFVVQLQDPREPRRQATQMLKLQNLVIPWAPENLTLHKLSESQLELNWNNRFLNHCLEHLVQYRTDWDHSWTEQSVDYRHKFSLPSVDGQKRYTFRVRSRFNPLCGSAQHWSEWSHPIHWGSNTSKENPFLFALEAVVISVGSMGLIISLLCVYFWLERTMPRIPTLKNLEDLVTEYHGNFSAWSGVSKGLAESLQPDYSERLCLVSEIPPKGGALGEGPGASPCNQHSPYWAPPCYTLKPET

SEQ ID NO: 64 - DNA, 258 bp, Artificial Sequence
  gamma chain intracellular region
gaacggacgatgccccgaattcccaccctgaagaacctagaggatcttgttactgaataccacgggaacttttcggcctggagtggtgtgtctaagggactggctgagagtctgcagccagactacagtgaacgactctgcctcgtcagtgagattcccccaaaaggaggggcccttggggaggggcctggggcctccccatgcaaccagcatagcccctactgggcccccccatgttacaccctaaagcctgaaacc

SEQ ID NO: 65 - protein, 86 aa, Artificial Sequence
  gamma chain intracellular region
ERTMPRIPTLKNLEDLVTEYHGNFSAWSGVSKGLAESLQPDYSERLCLVSEIPPKGGALGEGPGASPCNQHSPYWAPPCYTLKPET

SEQ ID NO: 66 - protein, 18 aa, Artificial Sequence
  linker
GSTSGSGKPGSGEGSTKG

SEQ ID NO: 67 - protein, 15 aa, Artificial Sequence
  linker
GGGGSGGGGSGGGGS

SEQ ID NO: 68 - protein, 18 aa, Artificial Sequence
  PDL1 signal peptide
MRIFAVFIFMTYWHLLNA

SEQ ID NO: 69 - protein, 223 aa, Artificial sequence
  PDL1 extracellular region
FTVTVPKDLYVVEYGSNMTIECKFPVEKQLDLAALIVYWEMEDKNIIQFVHGEEDLKVQHSSYRQRARLLKDQLSLGNAALQITDVKLQDAGVYRCMISYGGADYKRITVKVNAPYNKINQRILVVDPVTSEHELTCQAEGYPKAEVIWTSSDHQVLSGKTTTTNSKREEKLFNVTSTLRINTTTNEIFYCTFRRLDPEENHTAELVIPELPLAHPPNERTHL

SEQ ID NO: 70 - protein, 20 aa, Artificial Sequence
  PDL1 transmembrane domain
VILGAILLCLGVALTFIFRL

SEQ ID NO: 71 - protein, 246 aa, Artificial sequence
  KIR scFv
QVQLVQSGAEVKKPGSSVKVSCKASGGTFSFYAISWVRQAPGQGLEWMGGFIPIFGAANYAQKFQGRVTITADESTSTAYMELSSLRSDDTAVYYCARIPSGSYYYDYDMDVWGQGTTVTVSSGGGGSGGGGSGGGGSEIVLTQSPVTLSLSPGERATLSCRASQSVSSYLAWYQQKPGQAPRLLIYDASNRATGIPARFSGSGSGTDFTLTISSLEPEDFAVYYCQQRSNWMYTFGQGTKLEIKR

SEQ ID NO: 72 - protein, 243 aa, Artificial sequence
  LIR1 scFv-1
QVTLKESGPGILKPSQTLSLTCSFSGFSLSTSGLGVGWIRQPSGKGLEWLAHIWWDDDKYYLPSLKSQLTISKDTSRNQVFLKITSVDTADTATYYCARTELGRGDYWGQGTSVAVSSGSTSGSGKPGSGEGSTKGDILLTQSPAILSVSPGERVSFSCRASQSIGTNIHWYQQRTNGSPRLLIKYASESISGIPSRFSGSGSGTDFTLTINSVESEDIADYYCQQSYSWPYTFGGGTKLEIK

SEQ ID NO: 73 - protein, 244 aa, Artificial sequence
  LIR1 scFv-2
DIVMTQSHKFMSTSVGDRVSITCKASQDVSTAVAWYQQKPGQSPKLLIYSASYRYTGVPDRFTGSGSGTDFTFTISSVQAEDLALYYCQQHYSPPWTFGGGTKLEIKRGGGGSGGGGSGGGGSEVQLQQSGTVLPRPGASVKMSCKASGYSFTNYWMHWVKQRPGQGLEWIGAIYPGNSDTSYNQKFEGKAKLTAVTSASTAYMELSSLTNEDSAVYYCTTYDGYYSAWFAYWGQGTLVTVSAA

SEQ ID NO: 74 - protein, 356 aa, Artificial sequence
  E- cadherin EC1-EC2
WLCQEPEPCHPGFDAESYTFTVPRRHLERGRVLGRVNFEDCTGRQRTAYFSLDTRFKVGTDGVITVKRPLRFHNPQIHFLVYAWDSTYRKFSTKVTLNTVGHHHRPPPHQASVSGIQAELLTFPNSSPGLRRQKRDWVIPPISCPENEKGPFPKNLVQIKSNKDKEGKVFYSITGQGADTPPVGVFIIERETGWLKVTEPLDRERIATYTLFSHAVSSNGNAVEDPMEILITVTDQNDNKPEFTQEVFKGSVMEGALPGTSVMEVTATDADDDVNTYNAAIAYTILSQDPELPDKNMFTINRNTGVISVVTTGLDRESFPTYTLVVQAADLQGEGLSTTATAVITVTDTNDNPPIF

SEQ ID NO: 75 - protein, 9 aa, Artificial sequence
  Presenting peptide
VMAPRTLIL

SEQ ID NO: 76 - DNA, 297 bp, Artificial sequence
  B2M with synonymous mutation
atccagaggaccccgaagatccaggtttattctcggcatcctgccgaaaatggaaaaagcaattttctcaactgttatgtgtctggatttcacccatctgacatagaggttgaccttcttaagaatggcgagagaatcgagaaggtcgaacattcagacttgagcttcagcaaggattggagcttttatcttctttattatactgaatttactcccactgaaaaggatgaatacgcctgcagggtaaaccatgtaacactcagtcagccaaagatcgtaaaatgggaccgagacatg

SEQ ID NO: 77 - protein, 99 aa, Artificial sequence [sequence omitted]

SEQ ID NO: 78 - protein, 284 aa, Artificial sequence
  HLA-E extracellular domain
GSHSLKYFHTSVSRPGRGEPRFISVGYVDDTQFVRFDNDAASPRMVPRAPWMEQEGSEYWDRETRSARDTAQIFRVNLRTLRGCYNQSEAGSHTLQWMHGCELGPDGRFLRGYEQFAYDGKDYLTLNEDLRSWTAVDTAAQISEQKSNDASEAEHQRAYLEDTCVEWLHKYLEKGKETLLHLEPPKTHVTHHPISDHEATLRCWALGFYPAEITLTWQQDGEGHTQDTELVETRPAGDGTFQKWAAVVVPSGEEQRYTCHVQHEGLPEPVTLRWKPASQPTIPI

SEQ ID NO: 79 - protein, 283 aa, Artificial sequence
  HLA-G extracellular domain
GSHSMRYFSAAVSRPGRGEPRFIAMGYVDDTQFVRFDSDSACPRMEPRAPWVEQEGPEYWEEETRNTKAHAQTDRMNLQTLRGYYNQSEASSHTLQWMIGCDLGSDGRLLRGYEQYAYDGKDYLALNEDLRSWTAADTAAQISKRKCEAANVAEQRRAYLEGTCVEWLHRYLENGKEMLQRADPPKTHVTHHPVFDYEATLRCWALGFYPAEIILTWQRDGEDQTQDVELVETRPAGDGTFQKWAAVVVPSGEEQRYTCHVQHEGLPEPLMLRWKQSSLPTIP

SEQ ID NO: 80 - protein, 244 aa, Artificial sequence
  NKG2A scFv
EIVLTQSPATLSLSPGERATLSCSASSSVSSYIYWYQQKPGQAPRLLIYLTSNLASGIPARFSGSGSGTDFTLTISSLEPEDFAVYYCQQWSGNPYTFGQGTKLEIKGSTSGSGKPGSGEGSTKGEVQLVESGGGLVKPGGSLRLSCAASGFTFSSYAKSWVRQAPGKGLEWVSEISSGGSYTYYADSVKGRFTISRDNAKNSLYLQMNSLRAEDTAVYYCARHGDYPRFFDVWGQGTTVTVSS

SEQ ID NO: 81 - protein, 241 aa, Artificial Sequence
  SIGLEC7 scFv
DIQMTQTTSSLSASLGDRVTISCSASQGITNYLNWYQQKPDGTVKLLIYYTSILHSGVPSRFSGSGSGTDYSLTISNLEPEDIATYYCQQYSKPPYTFGGGTKLEIKGGGGSGGGGSGGGGSEVKLEESGGGLVQPGGSMKVSCVASGFTFSNYWMNWVRQSPEKGLEWVAQIRLKSDNYATHYAESVKGRFTISRDDSKSSVYLQMNNLRAEDTGIYYCTEGDYDIFAYWGQGTLVTVSA

SEQ ID NO: 82 - protein, 237 aa, Artificial Sequence
  SIGLEC7/9 scFv
DVQLQESGPLVKPSQSLSLTCTVTGYSITGGFAWNWIRQFPGNTLEWMGYIGYGGSTSYNPSLNSRISITRDTSKNHFFLQFNSVTTDDSATYYCARGDYLFAYWGQGTLVTVSAGGGGSGGGGSGGGGSDIVMTQSHKFMSTSVGDRVSITCKASQDVNTAVAWYQQKPGQSPKLLIYSASYRYTGVPDRFTGSGSGTDFTFTISSVQAEDLAVYYCQQHYSTPRTFGGGTKLEIK

SEQ ID NO: 83 - protein, 241 aa, Artificial Sequence
  KLRG1 scFv
QVQLQQPGAEFVKPGASVKLSCKASGYTFTSYWIHWMKQRPGQGLEWIGNIYPGRSNNNYNEKFKNRATLTVDTSSSTAYMQFRSLTSDDSAVYYCARDATVEPLPYWGQGTLVTVSAGGGGSGGGGSGGGGSENVLTQSPAIMSASPGEKVTMTCRASSSVSSNYLHWYQQKSGASPKIWIYSTSNLASAVPARFSGSGSGTSYSLTISSVEAEDAATYYCQQYSGYPLTFGGGTKLEIK